European Patent Application EP 4 317 435 A1, published February 7, 2024. Title: Stable Multispecific Antibody and Use Thereof. Applicant: Daiichi Sankyo Company, Limited. The sequence listing filed with the application follows.

SEQUENCE LISTING (49 sequences)

SEQ ID NO: 1 - protein, 216 aa, Artificial
  Amino acid sequence of C3E-7085-Fab
EVQLVESGGGLVQPGGSLRLSCAASGVTFNYYGMSWIRQAPGKGLEWVASITRSGGRIYYPDSVKGRFTISRENTQKTLYLQMNSLRAEDTAVYYCTLDGRDGWVAYWGQGTLVTVSSASTKGPSVFPLAPSSKSTSGGTAALGCLVKDYFPEPVTVSWNSGALTSGVHTFPAVLQSSGLYSLSSVVTVPSSSLGTQTYICNVNHKPSNTKVDKRV

SEQ ID NO: 2 - protein, 213 aa, Artificial
  Amino acid sequence of C3E-7085-LC
NFMLTQPSSVSGVPGQRVTISCTGNTGNIGSNYVNWYQQLPGTAPKLLIYRDDKRPSGVPDRFSGSKSGTSASLAITGFQAEDEADYYCQSYSSGFIFGGGTKLTVLGQPKAAPSVTLFPPSSEELQANKATLVCLISDFYPGAVTVAWKADSSPVKAGVETTTPSKQSNNKYAASSYLSLTPEQWKSHRSYSCQVTHEGSTVEKTVAPTECS

SEQ ID NO: 3 - protein, 240 aa, Artificial
  Amino acid sequence of C3E-7096
EVQLVESGGGLVQPGGSLRLSCAASGVTFNYYGMSWIRQAPGKGLEWVASITRSGGRIYYPDSVKGRFTISRENTQKTLYLQMNSLRAEDTAVYYCTLDGRDGWVAYWGCGTLVTVSSGGGGSGGGGSGGGGSNFMLTQPSSVSGVPGQRVTISCTGNTGNIGSNYVNWYQQLPGTCPKLLIYRDDKRPSGVPDRFSGSKSGTSASLAITGFQAEDEADYYCQSYSSGFIFGGGTKLTVL

SEQ ID NO: 4 - DNA, 738 bp, Artificial
  Full-length nucleotide sequence of HC_h
atgaagcacctctggttctttctcctgttggtggctgcaccaagatgggtcctgagcgacaagacgcacacttgccctccgtgtccagctcccgaagctgcaggaggtcccagcgttttcctgtttcctccaaagcccaaagacaccctgatgatctccaggactcccgaggtgacctgtgtagttgtcgacgttagccatgaggatcccgaggtcaagtttaactggtatgtcgacggagttgaagtccacaatgccaagaccaaaccacgagaagagcagtacaatagcacatatcgcgtagtgtctgtactgaccgtgttgcatcaggattggcttaatgggaaggagtacaagtgcaaagtgagcaacaaagcccttccggcgcccatagagaaaaccatcagcaaggcaaaggggcaacctcgggaacctcaggtctgcacactgccaccttctcgtgatgagctgactaagaaccaggtgtcactgtcctgtgccgtgaaaggcttttacccctccgacattgccgtggaatgggagtcaaatggtcagcctgagaacaactacaagactacaccgccagtgctcgattcagatggctctttcttcctggtttccaagctgacagtggacaaatccagatggcaacagggcaatgtgttcagctgcagtgtgatgcatgaagcccttcacaaccactatacgcagaaaagtctgagtctctctcctggaaaa

SEQ ID NO: 5 - DNA, 1482 bp, Artificial
  Full-length nucleotide sequence of C3E-7085-HC-k
atgaagcatctctggtttttcttgctgctcgtcgctgcacctcgatgggtgctgtcaggcgaagtccagctggttgaatctggcggtggcctggtgcaacctggagggtctttgagactgagttgtgccgcatcaggagtcaccttcaactactatggcatgtcatggatacgccaagctcccgggaaagggctcgaatgggtcgcatcaatcactcggtctggggggagaatctactatccagactcagtcaagggccgctttaccatcagccgtgagaatacccagaaaacgctgtacctacagatgaactcccttcgggcagaggacactgccgtgtactactgtacactggatgggcgagatgggtgggttgcctattggggccaaggtactcttgtgactgtgtcttcgggaggcggcggttccggtggtggtggttccggaggaggaggaagcaacttcatgctgacacagccgtcttccgtatctggcgtaccaggtcaacgcgtgaccatttcttgcaccggcaatacagggaacattggcagcaactatgtgaactggtatcagcagcttcccggaactgctcctaaactcctgatatacagggatgataagcggccttctggggtccctgatcggtttagtggctccaaaagcggaacctcggcgagcctggcaatcacaggctttcaggctgaggatgaggccgactattattgccagagttatagtagcggattcatctttggcgggggcacgaagttaaccgtgcttggtggagagcccaaaagcgccgacaagacccacacctgtccaccttgtcccgctccagaagccgctggggggccttccgtctttctctttcccccgaaacccaaagacacactgatgatctccagaacacccgaagtaacctgcgttgtggttgacgtatcccacgaagatcccgaagtgaagttcaattggtacgtggacggcgttgaggtgcacaatgccaaaacaaagcctagggaggaacagtacaattcgacatatagggtagtgtcagtcctgacagtgttacaccaggactggttgaacgggaaagagtacaagtgcaaggtgagcaacaaagcgcttccagcgccaattgagaagacgatttccaaagccaaaggacagccgagggaaccgcaggtctacaccttacccccatgcagagacgagttgaccaagaatcaggtgagtctatggtgcctcgtgaagggcttctatcccagcgatattgccgtcgagtgggaatctaatggccaaccagagaacaactacaagactacgccacccgttctggacagtgatgggagcttcttcctatactccaagctcactgtggacaagtcacgttggcaacagggaaatgttttcagttgtagcgtgatgcatgaggccttgcataatcactacactcagaaaagcctgtccctgtcacctggaaag

SEQ ID NO: 6 - DNA, 1401 bp, Artificial
  Full-length nucleotide sequence of C3E-7085-Fab-HC-k
atgaaacatctctggttctttctgctgctggtagccgcccctagatgggtcctcagtgaggttcagcttgtagagtccggcggcggcttggtgcagcccggaggttccctccggctttcttgcgctgcttcaggagttacgttcaattactatgggatgtcctggataaggcaggctcccggtaaggggttggaatgggtggccagtattacccgcagtggaggaagaatctactatccggattctgtgaaaggacggttcactatcagcagagaaaatacacagaaaaccctttatctccagatgaactcccttcgtgccgaggataccgctgtgtactactgcacactggatggccgagatgggtgggtagcctactggggtcaaggaacgcttgtgacagtttcctcagccagcactaagggaccaagcgtctttccgttggcacccagcagcaaaagtactagcggcggcacagctgcactgggctgcctggtgaaggactatttccctgaacccgtcaccgtgtcctggaactccggtgccttgacttccggtgttcacacattccccgcagtgctccagagttccgggctctactcactgtcatctgtggtcaccgtgcctagctcaagtctggggacccaaacttacatctgcaatgtgaaccataagcctagtaacaccaaagtcgacaaacgcgtcgagcccaagtcatgcgacaagacccacacatgtccaccttgtcccgcacctgaggcggctggtggcccatccgtgtttctgtttccaccaaagcctaaagacaccctgatgattagtcgaacaccagaggtgacttgcgttgtcgtcgatgtgtcacacgaagatccggaggtaaagttcaactggtacgtcgatggggtggaggttcataacgccaagactaagccaagagaagagcagtacaactctacgtatagggtggtaagcgtactgacagtgttgcaccaggattggctcaatggcaaggaatacaagtgtaaggtgtctaataaggcgctgcctgcgccaattgagaaaacgatctctaaggccaaagggcaaccaagggagccccaagtctataccctgcctccgtgtcgggacgaactgactaagaaccaagtgagcctctggtgcctggtcaaaggcttttatcccagcgacatagcagtggaatgggagagcaatgggcagccagagaacaactacaagaccacacctcccgttctggactctgacggatcattctttctgtattccaaactgacagttgacaagtctcgctggcagcagggaaatgtgttcagctgtagcgtgatgcatgaagccctgcacaatcactatacccagaaaagcctgagcctgtctcccggcaaa

SEQ ID NO: 7 - DNA, 699 bp, Artificial
  Full-length nucleotide sequence of C3E-7085-LC
atggttctgcagactcaggtgttcatttcccttctgctgtggattagtggggcatatgggaatttcatgctgactcagccaagctccgtaagcggagtacccggccaaagagtcacaatcagttgcactggtaacaccggtaatatcggctctaactacgtgaattggtaccagcagttgccaggaacagcacccaaactcctgatctaccgcgatgacaagcgaccatctggcgtgcctgatcggtttagcgggagcaaaagtggcacaagtgcctcattggccataacggggttccaggcggaggatgaagcagactactattgccagtcctactcctctggcttcatctttggcggagggaccaagctcaccgtgcttggacaacccaaagcagctccatcagtgaccctgtttcctccttcttctgaggagctgcaggccaataaggccacactggtgtgtctcattagcgacttttatccgggtgcggtcactgtggcctggaaagccgactcaagtccggttaaggctggagttgagacaaccacaccctctaagcagagcaacaacaagtatgctgcctcaagctacctctcactgacccctgagcagtggaaatcccataggagctattcctgccaagtcacccacgaaggctccaccgtcgaaaagactgtggctcccacggaatgtagc

SEQ ID NO: 8 - DNA, 1482 bp, Artificial
  Full-length nucleotide sequence of C3E-7096-HC-k
atgaagcacctgtggttttttctgttactcgttgctgctcccagatgggtcttgagcggagaagtacagcttgtagagtcaggaggaggactggtacaaccaggtggctcgttacggctcagttgcgcagcctccggtgtgactttcaactactacggcatgagctggatacggcaagcgcctggaaaggggctcgaatgggtagcctccataacacggagtgggggtcgcatttactaccccgattctgtcaaaggccgcttcacaatcagcagagaaaacacgcagaaaacattgtacctccagatgaatagccttagggccgaagatacggcagtctactattgcaccctggatggcagggacggttgggttgcctattggggttgtggcaccttagtgaccgtatcctctggaggaggcggcagtggaggagggggatcagggggtggagggagtaacttcatgcttacacagccaagttctgtttcaggtgttcctgggcagagggttaccatctcttgcacagggaatacaggcaacattggcagcaactatgtgaattggtatcagcagctaccaggcacgtgtccgaaactgttgatctatcgggatgacaaaagaccgtccggagtgcctgatcgcttttccggctctaaatccgggacttcagcgagtttggccattactgggtttcaggcagaagatgaggccgactactactgccagagctactctagcgggttcatctttggcggtgggaccaagctgactgtgctgggcggcgaacccaaatccgccgacaaaacccacacttgtccgccatgtcctgctccagaggcagctggtggcccctctgtctttctgtttccccctaagcccaaggacacactgatgatttcgcgtactccagaggtgacgtgtgtggtggtggatgtgtctcatgaagatcccgaggtgaagttcaattggtatgtggacggagtggaagtccacaacgctaagacaaagcctagggaagagcagtataactccacctacagagtcgttagcgtgctgaccgtgctccatcaagactggctcaatggcaaggagtacaagtgcaaagtctccaataaggcccttcctgctcccatcgagaaaaccatctcaaaggcgaaaggacaaccccgagaacctcaggtctataccctaccaccctgtcgtgacgagctgactaaaaatcaggtgtcactgtggtgcctagtcaaagggttctatccctctgacattgccgtggagtgggagagcaatggccagccagagaacaactacaagaccacacctccagtcctggactcggatggctccttcttcctgtacagcaagctcaccgttgacaagtcacgatggcagcaagggaatgtgttctcatgcagcgtgatgcatgaggcacttcacaaccactatactcagaagtccctgagcttgagtccggggaaa

SEQ ID NO: 9 - protein, 246 aa, Artificial
  Full-length amino acid sequence of HC_h
MKHLWFFLLLVAAPRWVLSDKTHTCPPCPAPEAAGGPSVFLFPPKPKDTLMISRTPEVTCVVVDVSHEDPEVKFNWYVDGVEVHNAKTKPREEQYNSTYRVVSVLTVLHQDWLNGKEYKCKVSNKALPAPIEKTISKAKGQPREPQVCTLPPSRDELTKNQVSLSCAVKGFYPSDIAVEWESNGQPENNYKTTPPVLDSDGSFFLVSKLTVDKSRWQQGNVFSCSVMHEALHNHYTQKSLSLSPGK

SEQ ID NO: 10 - protein, 494 aa, Artificial
  Full-length amino acid sequence of C3E-7085-HC-k
MKHLWFFLLLVAAPRWVLSGEVQLVESGGGLVQPGGSLRLSCAASGVTFNYYGMSWIRQAPGKGLEWVASITRSGGRIYYPDSVKGRFTISRENTQKTLYLQMNSLRAEDTAVYYCTLDGRDGWVAYWGQGTLVTVSSGGGGSGGGGSGGGGSNFMLTQPSSVSGVPGQRVTISCTGNTGNIGSNYVNWYQQLPGTAPKLLIYRDDKRPSGVPDRFSGSKSGTSASLAITGFQAEDEADYYCQSYSSGFIFGGGTKLTVLGGEPKSADKTHTCPPCPAPEAAGGPSVFLFPPKPKDTLMISRTPEVTCVVVDVSHEDPEVKFNWYVDGVEVHNAKTKPREEQYNSTYRVVSVLTVLHQDWLNGKEYKCKVSNKALPAPIEKTISKAKGQPREPQVYTLPPCRDELTKNQVSLWCLVKGFYPSDIAVEWESNGQPENNYKTTPPVLDSDGSFFLYSKLTVDKSRWQQGNVFSCSVMHEALHNHYTQKSLSLSPGK

SEQ ID NO: 11 - protein, 467 aa, Artificial
  Full-length amino acid sequence of C3E-7085-Fab-HC-k
MKHLWFFLLLVAAPRWVLSEVQLVESGGGLVQPGGSLRLSCAASGVTFNYYGMSWIRQAPGKGLEWVASITRSGGRIYYPDSVKGRFTISRENTQKTLYLQMNSLRAEDTAVYYCTLDGRDGWVAYWGQGTLVTVSSASTKGPSVFPLAPSSKSTSGGTAALGCLVKDYFPEPVTVSWNSGALTSGVHTFPAVLQSSGLYSLSSVVTVPSSSLGTQTYICNVNHKPSNTKVDKRVEPKSCDKTHTCPPCPAPEAAGGPSVFLFPPKPKDTLMISRTPEVTCVVVDVSHEDPEVKFNWYVDGVEVHNAKTKPREEQYNSTYRVVSVLTVLHQDWLNGKEYKCKVSNKALPAPIEKTISKAKGQPREPQVYTLPPCRDELTKNQVSLWCLVKGFYPSDIAVEWESNGQPENNYKTTPPVLDSDGSFFLYSKLTVDKSRWQQGNVFSCSVMHEALHNHYTQKSLSLSPGK

SEQ ID NO: 12 - protein, 233 aa, Artificial
  Full-length amino acid sequence of C3E-7085-LC
MVLQTQVFISLLLWISGAYGNFMLTQPSSVSGVPGQRVTISCTGNTGNIGSNYVNWYQQLPGTAPKLLIYRDDKRPSGVPDRFSGSKSGTSASLAITGFQAEDEADYYCQSYSSGFIFGGGTKLTVLGQPKAAPSVTLFPPSSEELQANKATLVCLISDFYPGAVTVAWKADSSPVKAGVETTTPSKQSNNKYAASSYLSLTPEQWKSHRSYSCQVTHEGSTVEKTVAPTECS

SEQ ID NO: 13 - protein, 494 aa, Artificial
  Full-length amino acid sequence of C3E-7096-HC-k
MKHLWFFLLLVAAPRWVLSGEVQLVESGGGLVQPGGSLRLSCAASGVTFNYYGMSWIRQAPGKGLEWVASITRSGGRIYYPDSVKGRFTISRENTQKTLYLQMNSLRAEDTAVYYCTLDGRDGWVAYWGCGTLVTVSSGGGGSGGGGSGGGGSNFMLTQPSSVSGVPGQRVTISCTGNTGNIGSNYVNWYQQLPGTCPKLLIYRDDKRPSGVPDRFSGSKSGTSASLAITGFQAEDEADYYCQSYSSGFIFGGGTKLTVLGGEPKSADKTHTCPPCPAPEAAGGPSVFLFPPKPKDTLMISRTPEVTCVVVDVSHEDPEVKFNWYVDGVEVHNAKTKPREEQYNSTYRVVSVLTVLHQDWLNGKEYKCKVSNKALPAPIEKTISKAKGQPREPQVYTLPPCRDELTKNQVSLWCLVKGFYPSDIAVEWESNGQPENNYKTTPPVLDSDGSFFLYSKLTVDKSRWQQGNVFSCSVMHEALHNHYTQKSLSLSPGK

SEQ ID NO: 14 - DNA, 2232 bp, Artificial
  Full-length nucleotide sequence of TX3-0001-HC_k
atgaagcacctgtggttctttctgctgcttgtggccgcaccacggtgggtgctgtcaggtcaggtgcagttagtgcagtcaggcgcagaagtaaagaaaccaggagcttcagtgaaggtcagttgcaaggcttctgggtatacgttcactaccgcagggatgcagtgggtgcgccaagctccagggcagggactggagtggatggggtggattaatacccatagcggggtcccaaagtacgcggaagatttcaaaggcagagtcaccatttctgccgatacgagcacatcgacagcatacctccagcttagttccttgaagagtgaggacacagctgtatactactgcgccagatccggttttggtagcagttactggtacttcgacgtgtggggccaaggcacactcgtgactgtatcctcaggagggggaggttccggtggcggcggctctggaggaggcggaagcgacattcagatgacccagtctcccagtagccttagcgccagtgttggcgatagagtgacaatcacctgtaaagcctctcaggacgtgtcgacagcagtggcatggtatcagcagaaacccggaaaggctcccaagctactgatatattccgcgtcgtatcggtacacaggggtaccatctcgcttctcgggttccggcagcggcaccgactttaccctcacaattagctctttacagcccgaagacttcgcagtgtattattgccagcaacactatatcaccccgctgacttttgggcagggtacgaagcttgagatcaaacggactggcgggggtgggtctgaggtccagctggttgaatccggcgggggattagtgcagccaggcggttcactgaggttgagctgtgcagcctctggagtcacgtttaactactatggcatgtcctggattagacaagccccaggcaaaggcctggagtgggtagcctctatcacccgaagcggtggacgcatctattacccagatagcgtgaagggccggttcacaatcagtagagagaacacccagaagacactgtacctacaaatgaacagcctaagagccgaggataccgcggtgtactactgtacactcgatggaagggatgggtgggtggcttactgggggcaggggactctcgtcaccgttagtagtggcggtggcggtagcggaggaggaggtagcggcggaggtgggtcaaatttcatgctcacacagcccagctcagtctccggggtacctggccagcgtgtgactatctcctgcactggcaataccggaaacataggaagcaattacgtaaactggtatcaacagcttccgggcactgcccctaaactcctgatttaccgcgatgataaaaggccttccggcgtcccagacaggtttagtggctcgaaatccgggacaagcgccagtttggcaattaccggatttcaagccgaagatgaagctgactactactgccagtcctattcatcagggttcatatttggcggtggaactaaactgaccgtccttggaggggaacccaagagcgccgacaaaacacacacttgtcctccgtgtcccgcgcccgaagctgctggggggcccagtgtgttcctatttccccccaagccaaaggacacgttgatgatctctcgtacccctgaggtcacgtgcgttgtggttgacgtctcccacgaagatcccgaggtgaaattcaactggtatgtggacggcgttgaggtgcacaatgccaaaactaagccgagggaagagcagtacaactctacctatcgggtggtgtctgttttgacagttctccatcaggactggctgaatggaaaagagtacaagtgcaaggtgagtaacaaagctctgccagcccctatcgagaaaaccatctccaaggccaaaggccaaccacgagagcctcaagtttacaccctccctccttgtcgagacgagctgaccaagaaccaagtctccttatggtgtctcgtgaagggattttatccctcagacattgccgtggagtgggaatctaatggccagcctgagaacaattataagacaactcctcctgtccttgattccgatggctcctttttcctgtactctaagttgactgtcgacaagtcacgctggcagcaggggaatgttttctcttgcagcgttatgcatgaagctctgcataaccactatactcagaaaagcctgtcactgtcaccggggaag

SEQ ID NO: 15 - DNA, 2232 bp, Artificial
  Full-length nucleotide sequence of TX3-0003-HC_k
atgaagcatctctggtttttcctgctcctggtggcggctccaagatgggtgttgagcggtcaggtgcaactggtgcagtcaggagcggaggtcaagaaacccggcgcgagtgtcaaagtgagttgcaaagcttccggatatactttcactaccgctggaatgcaatgggtgagacaagcaccagggcaaggcttggaatggatgggctggatcaacacacactctggggttcccaagtatgccgaagactttaagggtagggtcaccatatcagccgatacatcaacctcgaccgcatacctccagctgtcctcccttaagagcgaggatactgctgtttactattgcgctaggtcaggattcggctcttcttactggtactttgatgtgtgggggcagggcacacttgtgacggtttcctctggcggcggcgggtcaggaggtggtggctctggagggggtggttcagacatccagatgacccagagtccttcctccttgagtgccagtgtaggcgacagagtcactattacctgcaaggcctctcaggacgtgtcgacagcggttgcatggtatcagcagaaacctgggaaggctccaaagctcctgatctactcagccagctatcggtacactggggtcccttctcgctttagcggctctggtagcgggaccgacttcacgcttaccatcagttccctgcaaccggaggactttgcagtgtactactgtcagcagcattacatcaccccactgacatttgggcaggggacaaagcttgagattaaacggacaggcggcggaggaagcgaggtgcagttagtggagagcggagggggtttagtccaaccgggcgggagcctccgtctgagctgtgctgcttccggcgttaccttcaactattatggaatgagctggatcaggcaagcccctggcaaaggtcttgaatgggttgcatctatcactcgatcagggggtcgcatttattacccggatagcgttaaaggcaggttcacaatctctcgggagaacactcagaaaaccctctatctacagatgaactctttacgggccgaagatacagccgtctattattgcactctagatggtcgagatggctgggtcgcctattgggggtgtggaaccttggtcactgttagcagtggaggaggaggatcaggagggggcgggtccggcggtgggggtagcaatttcatgctgacacaaccttcttcagtatctggcgtgccaggacagcgcgtcaccatctcttgtaccggcaatacaggtaacattggctccaattacgtgaattggtaccagcagcttcctggcacctgccctaagctgctgatttaccgggacgataagaggccctcgggggtgcccgaccgtttctcgggaagcaagtccgggacatccgcctcacttgccattacggggtttcaggccgaggatgaagctgattactactgccagtcttactccagtggcttcatttttggcggaggcaccaagctgacagtgctaggcggagaacccaaaagtgcagacaagacgcatacttgccccccgtgtcctgctccagaagcagcaggaggaccctctgttttcctctttccacctaaacccaaggacactctgatgataagcagaacacctgaagtgacgtgtgttgtggtagatgtctcccatgaagatcccgaagtcaagttcaactggtacgtggacggcgtggaggtgcacaatgccaaaacgaagcccagagaggagcagtataactccacatacagagttgtgagcgtactgactgtattgcaccaagactggctgaatggtaaggagtacaagtgcaaggtgtcaaacaaagctctgcctgcacccatagagaaaaccatcagtaaggccaaagggcagccacgcgagccacaggtgtatactctgccaccatgccgagacgagctcactaagaatcaggtgagcttgtggtgtctcgtaaagggcttttacccctcggacattgccgtagagtgggaatccaatgggcaacccgagaacaattacaaaaccacaccgccagtgttagacagcgatggaagcttctttctctatagcaagctgaccgtcgacaaaagtcgctggcagcaggggaacgtcttcagttgttccgtgatgcacgaagccctacacaaccactatacccagaaatccctgtcactgagtcctggcaaa

SEQ ID NO: 16 - DNA, 2229 bp, Artificial
  Full-length nucleotide sequence of CX3-0001-HC_k
atgaagcacctgtggttctttctgctgctggtggccgctcctagatgggtgctgtctggacaggttcagctggttcagtctggcgccgaagtgaagaaacctggcgcctctgtgaaggtgtcctgcaaggcctctggctacgccttcagcaactacctgatcgagtgggtccgacaggcccctggacaaggacttgaatggatgggcgtgatcaaccctggcagcggcgtgaccaactacaacgagaagttcaagggcagagtgaccatcaccgccgacaccagcacaagcaccgcctacatggaactgagcagcctgagaagcgaggacaccgccgtgtactattgtgccagagccgaggcttggtttgcctattggggacagggcaccctggtcaccgttagctctggtggaggcggttcaggcggaggtggcagcggcggtggcgggagtgatattgtgatgacacagagccccgacagcctggccgtgtctcttggagaaagagccaccatcaactgcaagagcagccagagcctgctgtactccagcaaccagaagaactacctggcctggtatcagcagaagcccggccagcctcctaagctgctgatctactgggccagcaccagagaaagcggcgtgcccgatagattttctggctctggcagcggcaccgacttcaccctgacaatttctagcctgcaagccgaggacgtggccgtgtactactgccagagatattacggctacccctggacctttggccagggcaccaaggtggaaatcaagggaggcggaggatctgaagtgcagctggtggaatccggggggggcctggtgcagcctggggggagcctgagactgagttgtgccgcctctggggtgacatttaactactatggcatgtcttggatccgccaggcacctggaaagggcctggagtgggtggccagcatcactaggtccggcgggcgaatctactatcccgacagcgtcaagggcaggttcacaatttcccgcgagaacacacagaaaactctgtacctgcagatgaatagcctgagagccgaagatacagctgtgtactattgcactctggacggcagggatgggtgggtcgcctattgggggcagggaaccctggtgacagtcagctccggaggaggaggatctggcggaggaggcagtgggggaggcgggtcaaactttatgctcactcagccgtcctctgtttctggcgtacctggccaacgggtgaccattagctgtacgggtaataccgggaatatcgggtctaactacgtgaactggtatcagcagcttccagggacagctcccaagttgctgatctatcgcgacgacaaaagaccctcaggggtccctgaccgatttagtggcagcaaaagcggtacttccgcttccctggcgataaccggctttcaggccgaagatgaggcagactactattgccagtcatattccagcggcttcatcttcggaggcggaactaagctgacagtgttgggcggagaacccaagagcgcagacaagacccacacctgtcctccatgtcctgctccagaagctgcaggcggcccttccgtgtttctgttccctccaaagcctaaggacaccctgatgatcagccggacacctgaagtgacctgcgtggtggtggatgtgtcccacgaggatcccgaagtgaagttcaattggtacgtggacggcgtggaagtgcacaacgccaagaccaagcctagagaggaacagtacaacagcacctacagagtggtgtctgtgctgacagtgctgcaccaggactggctgaacggcaaagagtacaagtgcaaggtgtccaacaaggccctgcctgctcctatcgagaaaaccatcagcaaggccaagggccagcctagggaaccccaggtttacaccctgcctccatgcagggatgagctgaccaagaaccaggtgtccctgtggtgcctggttaagggcttctacccctccgatatcgccgtggaatgggagagcaatggccagccagagaacaactacaagacaacccctcctgtgctggactccgacggctcattcttcctgtacagcaagctgaccgtggacaagagcagatggcagcagggcaacgtgttcagctgcagcgtgatgcacgaggccctgcacaaccactacacacagaagtccctgtctctgagccccggcaaa

SEQ ID NO: 17 - DNA, 2229 bp, Artificial
  Full-length nucleotide sequence of p_CX3-0003-HC_k
atgaagcacctgtggttctttctgctgctggtggccgctcctagatgggtgctgtctggacaggttcagctggttcagtctggcgccgaagtgaagaaacctggcgcctctgtgaaggtgtcctgcaaggcctctggctacgccttcagcaactacctgatcgagtgggtccgacaggcccctggacaaggacttgaatggatgggcgtgatcaaccctggcagcggcgtgaccaactacaacgagaagttcaagggcagagtgaccatcaccgccgacaccagcacaagcaccgcctacatggaactgagcagcctgagaagcgaggacaccgccgtgtactattgtgccagagccgaggcttggtttgcctattggggacagggcaccctggtcaccgttagctctggtggaggcggttcaggcggaggtggcagcggcggtggcgggagtgatattgtgatgacacagagccccgacagcctggccgtgtctcttggagaaagagccaccatcaactgcaagagcagccagagcctgctgtactccagcaaccagaagaactacctggcctggtatcagcagaagcccggccagcctcctaagctgctgatctactgggccagcaccagagaaagcggcgtgcccgatagattttctggctctggcagcggcaccgacttcaccctgacaatttctagcctgcaagccgaggacgtggccgtgtactactgccagagatattacggctacccctggacctttggccagggcaccaaggtggaaatcaagggaggcggaggatctgaagtgcagctggtggaatccggggggggcctggtgcagcctggggggagcctgagactgagttgtgccgcctctggggtgacatttaactactatggcatgtcttggatccgccaggcacctggaaagggcctggagtgggtggccagcatcactaggtccggcgggcgaatctactatcccgacagcgtcaagggcaggttcacaatttcccgcgagaacacacagaaaactctgtacctgcagatgaatagcctgagagccgaagatacagctgtgtactattgcactctggacggcagggatgggtgggtcgcctattgggggtgtggaaccctggtgacagtcagctccggaggaggaggatctggcggaggaggcagtgggggaggcgggtcaaactttatgctcactcagccgtcctctgtttctggcgtacctggccaacgggtgaccattagctgtacgggtaataccgggaatatcgggtctaactacgtgaactggtatcagcagcttccagggacatgtcccaagttgctgatctatcgcgacgacaaaagaccctcaggggtccctgaccgatttagtggcagcaaaagcggtacttccgcttccctggcgataaccggctttcaggccgaagatgaggcagactactattgccagtcatattccagcggcttcatcttcggaggcggaactaagctgacagtgttgggcggagaacccaagagcgcagacaagacccacacctgtcctccatgtcctgctccagaagctgcaggcggcccttccgtgtttctgttccctccaaagcctaaggacaccctgatgatcagccggacacctgaagtgacctgcgtggtggtggatgtgtcccacgaggatcccgaagtgaagttcaattggtacgtggacggcgtggaagtgcacaacgccaagaccaagcctagagaggaacagtacaacagcacctacagagtggtgtctgtgctgacagtgctgcaccaggactggctgaacggcaaagagtacaagtgcaaggtgtccaacaaggccctgcctgctcctatcgagaaaaccatcagcaaggccaagggccagcctagggaaccccaggtttacaccctgcctccatgcagggatgagctgaccaagaaccaggtgtccctgtggtgcctggttaagggcttctacccctccgatatcgccgtggaatgggagagcaatggccagccagagaacaactacaagacaacccctcctgtgctggactccgacggctcattcttcctgtacagcaagctgaccgtggacaagagcagatggcagcagggcaacgtgttcagctgcagcgtgatgcacgaggccctgcacaaccactacacacagaagtccctgtctctgagccccggcaaa

SEQ ID NO: 18 - DNA, 2217 bp, Artificial
  Full-length nucleotide sequence of RX3-0001-HC_k
atgaagcacctgtggttctttctgctgctggtggccgctcctagatgggtgctgtctggacaggtgcagctggtgcagtctggcgccgaagtgaagaaaccaggcgccagcgtgaaggtgtcctgcaaggccagcggctacacctttaccggctactacatgcactgggtgcgccaggctccaggccagggactggaatggatgggccggatcaaccccaatagcggcggcaccaactacgcccagaaattccagggcagagtgaccatgacccgggacaccagcatcagcaccgcctacatggaactgagcggcctgagaagcgacgacaccgccgtgtactactgtgcctctggctctgtgcggcacccttggggacagggaacactcgtgaccgtgtccagcggtggaggcggttcaggcggaggtggcagcggcggtggcgggagtcagcctgtgctgacacagcctccaagcgcctctggcacacctggccagagagtgacaatcagctgcagcggcagcagaagcaacatcggcggcaacatcgtgtcctggtatcagcagttccccggcaccgcccctagactgctgacctacgccgacaaccagaggcctagcggcgtgcccgatagattcagcggctctaagagcggcaccagcgccagcctggccatctctggcctgcagtctgaggacgaggccgactactattgcgccgcctgggacgacagcctgaacggcgtggtgtttggcggaggcaccaagctgacagtgctgggaggcggaggatctgaagtgcagctggtggaatccggggggggcctggtgcagcctggggggagcctgagactgagttgtgccgcctctggggtgacatttaactactatggcatgtcttggatccgccaggcacctggaaagggcctggagtgggtggccagcatcactaggtccggcgggcgaatctactatcccgacagcgtcaagggcaggttcacaatttcccgcgagaacacacagaaaactctgtacctgcagatgaatagcctgagagccgaagatacagctgtgtactattgcactctggacggcagggatgggtgggtcgcctattgggggcagggaaccctggtgacagtcagctccggaggaggaggatctggcggaggaggcagtgggggaggcgggtcaaactttatgctcactcagccgtcctctgtttctggcgtacctggccaacgggtgaccattagctgtacgggtaataccgggaatatcgggtctaactacgtgaactggtatcagcagcttccagggacagctcccaagttgctgatctatcgcgacgacaaaagaccctcaggggtccctgaccgatttagtggcagcaaaagcggtacttccgcttccctggcgataaccggctttcaggccgaagatgaggcagactactattgccagtcatattccagcggcttcatcttcggaggcggaactaagctgacagtgttgggcggagaacccaagagcgcagacaagacccacacctgtcctccatgtcctgctccagaagctgcaggcggcccttccgtgtttctgttccctccaaagcctaaggacaccctgatgatcagccggacacctgaagtgacctgcgtggtggtggatgtgtcccacgaggatcccgaagtgaagttcaattggtacgtggacggcgtggaagtgcacaacgccaagaccaagcctagagaggaacagtacaacagcacctacagagtggtgtctgtgctgacagtgctgcaccaggactggctgaacggcaaagagtacaagtgcaaggtgtccaacaaggccctgcctgctcctatcgagaaaaccatcagcaaggccaagggccagcctagggaaccccaggtttacaccctgcctccatgcagggatgagctgaccaagaaccaggtgtccctgtggtgcctggttaagggcttctacccctccgatatcgccgtggaatgggagagcaatggccagccagagaacaactacaagacaacccctcctgtgctggactccgacggctcattcttcctgtacagcaagctgaccgtggacaagagcagatggcagcagggcaacgtgttcagctgcagcgtgatgcacgaggccctgcacaaccactacacacagaagtccctgtctctgagccccggcaaa

SEQ ID NO: 19 - DNA, 2217 bp, Artificial
  Full-length nucleotide sequence of RX3-0003-HC_k
atgaagcacctgtggttctttctgctgctggtggccgctcctagatgggtgctgtctggacaggtgcagctggtgcagtctggcgccgaagtgaagaaaccaggcgccagcgtgaaggtgtcctgcaaggccagcggctacacctttaccggctactacatgcactgggtgcgccaggctccaggccagggactggaatggatgggccggatcaaccccaatagcggcggcaccaactacgcccagaaattccagggcagagtgaccatgacccgggacaccagcatcagcaccgcctacatggaactgagcggcctgagaagcgacgacaccgccgtgtactactgtgcctctggctctgtgcggcacccttggggacagggaacactcgtgaccgtgtccagcggtggaggcggttcaggcggaggtggcagcggcggtggcgggagtcagcctgtgctgacacagcctccaagcgcctctggcacacctggccagagagtgacaatcagctgcagcggcagcagaagcaacatcggcggcaacatcgtgtcctggtatcagcagttccccggcaccgcccctagactgctgacctacgccgacaaccagaggcctagcggcgtgcccgatagattcagcggctctaagagcggcaccagcgccagcctggccatctctggcctgcagtctgaggacgaggccgactactattgcgccgcctgggacgacagcctgaacggcgtggtgtttggcggaggcaccaagctgacagtgctgggaggcggaggatctgaagtgcagctggtggaatccggggggggcctggtgcagcctggggggagcctgagactgagttgtgccgcctctggggtgacatttaactactatggcatgtcttggatccgccaggcacctggaaagggcctggagtgggtggccagcatcactaggtccggcgggcgaatctactatcccgacagcgtcaagggcaggttcacaatttcccgcgagaacacacagaaaactctgtacctgcagatgaatagcctgagagccgaagatacagctgtgtactattgcactctggacggcagggatgggtgggtcgcctattgggggtgtggaaccctggtgacagtcagctccggaggaggaggatctggcggaggaggcagtgggggaggcgggtcaaactttatgctcactcagccgtcctctgtttctggcgtacctggccaacgggtgaccattagctgtacgggtaataccgggaatatcgggtctaactacgtgaactggtatcagcagcttccagggacatgtcccaagttgctgatctatcgcgacgacaaaagaccctcaggggtccctgaccgatttagtggcagcaaaagcggtacttccgcttccctggcgataaccggctttcaggccgaagatgaggcagactactattgccagtcatattccagcggcttcatcttcggaggcggaactaagctgacagtgttgggcggagaacccaagagcgcagacaagacccacacctgtcctccatgtcctgctccagaagctgcaggcggcccttccgtgtttctgttccctccaaagcctaaggacaccctgatgatcagccggacacctgaagtgacctgcgtggtggtggatgtgtcccacgaggatcccgaagtgaagttcaattggtacgtggacggcgtggaagtgcacaacgccaagaccaagcctagagaggaacagtacaacagcacctacagagtggtgtctgtgctgacagtgctgcaccaggactggctgaacggcaaagagtacaagtgcaaggtgtccaacaaggccctgcctgctcctatcgagaaaaccatcagcaaggccaagggccagcctagggaaccccaggtttacaccctgcctccatgcagggatgagctgaccaagaaccaggtgtccctgtggtgcctggttaagggcttctacccctccgatatcgccgtggaatgggagagcaatggccagccagagaacaactacaagacaacccctcctgtgctggactccgacggctcattcttcctgtacagcaagctgaccgtggacaagagcagatggcagcagggcaacgtgttcagctgcagcgtgatgcacgaggccctgcacaaccactacacacagaagtccctgtctctgagccccggcaaa

SEQ ID NO: 20 - protein, 744 aa, Artificial
  Full-length amino acid sequence of TX3-0001-HC_k
MKHLWFFLLLVAAPRWVLSGQVQLVQSGAEVKKPGASVKVSCKASGYTFTTAGMQWVRQAPGQGLEWMGWINTHSGVPKYAEDFKGRVTISADTSTSTAYLQLSSLKSEDTAVYYCARSGFGSSYWYFDVWGQGTLVTVSSGGGGSGGGGSGGGGSDIQMTQSPSSLSASVGDRVTITCKASQDVSTAVAWYQQKPGKAPKLLIYSASYRYTGVPSRFSGSGSGTDFTLTISSLQPEDFAVYYCQQHYITPLTFGQGTKLEIKRTGGGGSEVQLVESGGGLVQPGGSLRLSCAASGVTFNYYGMSWIRQAPGKGLEWVASITRSGGRIYYPDSVKGRFTISRENTQKTLYLQMNSLRAEDTAVYYCTLDGRDGWVAYWGQGTLVTVSSGGGGSGGGGSGGGGSNFMLTQPSSVSGVPGQRVTISCTGNTGNIGSNYVNWYQQLPGTAPKLLIYRDDKRPSGVPDRFSGSKSGTSASLAITGFQAEDEADYYCQSYSSGFIFGGGTKLTVLGGEPKSADKTHTCPPCPAPEAAGGPSVFLFPPKPKDTLMISRTPEVTCVVVDVSHEDPEVKFNWYVDGVEVHNAKTKPREEQYNSTYRVVSVLTVLHQDWLNGKEYKCKVSNKALPAPIEKTISKAKGQPREPQVYTLPPCRDELTKNQVSLWCLVKGFYPSDIAVEWESNGQPENNYKTTPPVLDSDGSFFLYSKLTVDKSRWQQGNVFSCSVMHEALHNHYTQKSLSLSPGK

SEQ ID NO: 21 - protein, 744 aa, Artificial
  Full-length amino acid sequence of TX3-0003-HC_k
MKHLWFFLLLVAAPRWVLSGQVQLVQSGAEVKKPGASVKVSCKASGYTFTTAGMQWVRQAPGQGLEWMGWINTHSGVPKYAEDFKGRVTISADTSTSTAYLQLSSLKSEDTAVYYCARSGFGSSYWYFDVWGQGTLVTVSSGGGGSGGGGSGGGGSDIQMTQSPSSLSASVGDRVTITCKASQDVSTAVAWYQQKPGKAPKLLIYSASYRYTGVPSRFSGSGSGTDFTLTISSLQPEDFAVYYCQQHYITPLTFGQGTKLEIKRTGGGGSEVQLVESGGGLVQPGGSLRLSCAASGVTFNYYGMSWIRQAPGKGLEWVASITRSGGRIYYPDSVKGRFTISRENTQKTLYLQMNSLRAEDTAVYYCTLDGRDGWVAYWGCGTLVTVSSGGGGSGGGGSGGGGSNFMLTQPSSVSGVPGQRVTISCTGNTGNIGSNYVNWYQQLPGTCPKLLIYRDDKRPSGVPDRFSGSKSGTSASLAITGFQAEDEADYYCQSYSSGFIFGGGTKLTVLGGEPKSADKTHTCPPCPAPEAAGGPSVFLFPPKPKDTLMISRTPEVTCVVVDVSHEDPEVKFNWYVDGVEVHNAKTKPREEQYNSTYRVVSVLTVLHQDWLNGKEYKCKVSNKALPAPIEKTISKAKGQPREPQVYTLPPCRDELTKNQVSLWCLVKGFYPSDIAVEWESNGQPENNYKTTPPVLDSDGSFFLYSKLTVDKSRWQQGNVFSCSVMHEALHNHYTQKSLSLSPGK

SEQ ID NO: 22 - protein, 743 aa, Artificial
  Full-length amino acid sequence of CX3-0001-HC_k
MKHLWFFLLLVAAPRWVLSGQVQLVQSGAEVKKPGASVKVSCKASGYAFSNYLIEWVRQAPGQGLEWMGVINPGSGVTNYNEKFKGRVTITADTSTSTAYMELSSLRSEDTAVYYCARAEAWFAYWGQGTLVTVSSGGGGSGGGGSGGGGSDIVMTQSPDSLAVSLGERATINCKSSQSLLYSSNQKNYLAWYQQKPGQPPKLLIYWASTRESGVPDRFSGSGSGTDFTLTISSLQAEDVAVYYCQRYYGYPWTFGQGTKVEIKGGGGSEVQLVESGGGLVQPGGSLRLSCAASGVTFNYYGMSWIRQAPGKGLEWVASITRSGGRIYYPDSVKGRFTISRENTQKTLYLQMNSLRAEDTAVYYCTLDGRDGWVAYWGQGTLVTVSSGGGGSGGGGSGGGGSNFMLTQPSSVSGVPGQRVTISCTGNTGNIGSNYVNWYQQLPGTAPKLLIYRDDKRPSGVPDRFSGSKSGTSASLAITGFQAEDEADYYCQSYSSGFIFGGGTKLTVLGGEPKSADKTHTCPPCPAPEAAGGPSVFLFPPKPKDTLMISRTPEVTCVVVDVSHEDPEVKFNWYVDGVEVHNAKTKPREEQYNSTYRVVSVLTVLHQDWLNGKEYKCKVSNKALPAPIEKTISKAKGQPREPQVYTLPPCRDELTKNQVSLWCLVKGFYPSDIAVEWESNGQPENNYKTTPPVLDSDGSFFLYSKLTVDKSRWQQGNVFSCSVMHEALHNHYTQKSLSLSPGK

SEQ ID NO: 23 - protein, 743 aa, Artificial
  Full-length amino acid sequence of CX3-0003-HC_k
MKHLWFFLLLVAAPRWVLSGQVQLVQSGAEVKKPGASVKVSCKASGYAFSNYLIEWVRQAPGQGLEWMGVINPGSGVTNYNEKFKGRVTITADTSTSTAYMELSSLRSEDTAVYYCARAEAWFAYWGQGTLVTVSSGGGGSGGGGSGGGGSDIVMTQSPDSLAVSLGERATINCKSSQSLLYSSNQKNYLAWYQQKPGQPPKLLIYWASTRESGVPDRFSGSGSGTDFTLTISSLQAEDVAVYYCQRYYGYPWTFGQGTKVEIKGGGGSEVQLVESGGGLVQPGGSLRLSCAASGVTFNYYGMSWIRQAPGKGLEWVASITRSGGRIYYPDSVKGRFTISRENTQKTLYLQMNSLRAEDTAVYYCTLDGRDGWVAYWGCGTLVTVSSGGGGSGGGGSGGGGSNFMLTQPSSVSGVPGQRVTISCTGNTGNIGSNYVNWYQQLPGTCPKLLIYRDDKRPSGVPDRFSGSKSGTSASLAITGFQAEDEADYYCQSYSSGFIFGGGTKLTVLGGEPKSADKTHTCPPCPAPEAAGGPSVFLFPPKPKDTLMISRTPEVTCVVVDVSHEDPEVKFNWYVDGVEVHNAKTKPREEQYNSTYRVVSVLTVLHQDWLNGKEYKCKVSNKALPAPIEKTISKAKGQPREPQVYTLPPCRDELTKNQVSLWCLVKGFYPSDIAVEWESNGQPENNYKTTPPVLDSDGSFFLYSKLTVDKSRWQQGNVFSCSVMHEALHNHYTQKSLSLSPGK

SEQ ID NO: 24 - protein, 739 aa, Artificial
  Full-length amino acid sequence of RX3-0001-HC_k
MKHLWFFLLLVAAPRWVLSGQVQLVQSGAEVKKPGASVKVSCKASGYTFTGYYMHWVRQAPGQGLEWMGRINPNSGGTNYAQKFQGRVTMTRDTSISTAYMELSGLRSDDTAVYYCASGSVRHPWGQGTLVTVSSGGGGSGGGGSGGGGSQPVLTQPPSASGTPGQRVTISCSGSRSNIGGNIVSWYQQFPGTAPRLLTYADNQRPSGVPDRFSGSKSGTSASLAISGLQSEDEADYYCAAWDDSLNGVVFGGGTKLTVLGGGGSEVQLVESGGGLVQPGGSLRLSCAASGVTFNYYGMSWIRQAPGKGLEWVASITRSGGRIYYPDSVKGRFTISRENTQKTLYLQMNSLRAEDTAVYYCTLDGRDGWVAYWGQGTLVTVSSGGGGSGGGGSGGGGSNFMLTQPSSVSGVPGQRVTISCTGNTGNIGSNYVNWYQQLPGTAPKLLIYRDDKRPSGVPDRFSGSKSGTSASLAITGFQAEDEADYYCQSYSSGFIFGGGTKLTVLGGEPKSADKTHTCPPCPAPEAAGGPSVFLFPPKPKDTLMISRTPEVTCVVVDVSHEDPEVKFNWYVDGVEVHNAKTKPREEQYNSTYRVVSVLTVLHQDWLNGKEYKCKVSNKALPAPIEKTISKAKGQPREPQVYTLPPCRDELTKNQVSLWCLVKGFYPSDIAVEWESNGQPENNYKTTPPVLDSDGSFFLYSKLTVDKSRWQQGNVFSCSVMHEALHNHYTQKSLSLSPGK

SEQ ID NO: 25 - protein, 739 aa, Artificial
  Full-length amino acid sequence of RX3-0003-HC_k
MKHLWFFLLLVAAPRWVLSGQVQLVQSGAEVKKPGASVKVSCKASGYTFTGYYMHWVRQAPGQGLEWMGRINPNSGGTNYAQKFQGRVTMTRDTSISTAYMELSGLRSDDTAVYYCASGSVRHPWGQGTLVTVSSGGGGSGGGGSGGGGSQPVLTQPPSASGTPGQRVTISCSGSRSNIGGNIVSWYQQFPGTAPRLLTYADNQRPSGVPDRFSGSKSGTSASLAISGLQSEDEADYYCAAWDDSLNGVVFGGGTKLTVLGGGGSEVQLVESGGGLVQPGGSLRLSCAASGVTFNYYGMSWIRQAPGKGLEWVASITRSGGRIYYPDSVKGRFTISRENTQKTLYLQMNSLRAEDTAVYYCTLDGRDGWVAYWGCGTLVTVSSGGGGSGGGGSGGGGSNFMLTQPSSVSGVPGQRVTISCTGNTGNIGSNYVNWYQQLPGTCPKLLIYRDDKRPSGVPDRFSGSKSGTSASLAITGFQAEDEADYYCQSYSSGFIFGGGTKLTVLGGEPKSADKTHTCPPCPAPEAAGGPSVFLFPPKPKDTLMISRTPEVTCVVVDVSHEDPEVKFNWYVDGVEVHNAKTKPREEQYNSTYRVVSVLTVLHQDWLNGKEYKCKVSNKALPAPIEKTISKAKGQPREPQVYTLPPCRDELTKNQVSLWCLVKGFYPSDIAVEWESNGQPENNYKTTPPVLDSDGSFFLYSKLTVDKSRWQQGNVFSCSVMHEALHNHYTQKSLSLSPGK

SEQ ID NO: 26 - DNA, 2154 bp, Artificial
  Full-length nucleotide sequence of TX3-0002-HC_k
atgaagcacctgtggttctttctgctgctggtggccgctcctagatgggtgctgtctggacaggttcagctggtgcagtctggcgccgaagtgaaaaaacctggcgcctccgtgaaggtgtcctgcaaggctagcggctacacctttaccacagccggcatgcagtgggtccgacaggctcctggacaaggactcgagtggatgggctggatcaatacccacagcggcgtgcccaaatacgccgaggatttcaagggcagagtgaccatcagcgccgacaccagcacaagcacagcctacctgcagctgagcagcctgaagtctgaggacaccgccgtgtactactgtgccagaagcggctttggcagcagctactggtacttcgatgtgtggggccagggcaccctggtcacagtttctagcggaggcggaggatctggtggcggaggaagtggcggaggcggttctgatatccagatgacacagagccccagcagcctgtctgcctctgtgggagacagagtgacaattacatgcaaggccagccaggacgtgtccacagcagttgcttggtaccagcagaagcctggcaaggcccctaagctgctgatctacagcgccagctacagatacaccggcgtgccaagcagattttccggctctggcagcggcaccgatttcaccctgaccatatctagcctgcagccagaggacttcgccgtgtattattgccagcagcactacatcacccctctgacctttggccaggggaccaagctcgagatcaagagaacaggtggcggcggatctgaggtgcagctggttgaaagcggcggaggacttgttcagcctggcggatctctgagactgagctgtgctgctagcggcgtgaccttcaactactacggcatgagctggatccgccaagctccaggcaagggcctcgagtgggttgccagcattacaagatctggcggccgcatctactaccccgactctgtgaagggcagattcacaatcagccgcgagaacacccagaaaaccctgtacctgcagatgaactccctgagagccgaggatacagctgtgtactattgcaccctggacggcagagatggctgggttgcatattggggacagggaaccctcgtgaccgtgtcctctgcctctacaaagggccctagcgtgttccctctggctcctagcagcaagagcacaagcggaggaacagccgctctgggctgtctggtcaaggactactttcccgagcctgtgacagtgtcctggaactctggcgctctgacatccggcgtgcacacatttccagccgtgctgcaaagcagcggcctgtactctctgagcagcgtcgtgacagtgcctagcagctctctgggcacccagacctacatctgcaatgtgaaccacaagcctagcaacaccaaggtggacaagagagtggaacccaagagctgcgacaagacccacacctgtcctccatgtcctgcacctgaagctgctggcggcccttccgtgtttctgttccctccaaagcctaaggacaccctgatgatcagcagaacccctgaagtgacctgcgtggtggtggatgtgtctcacgaggacccagaagtgaagttcaattggtacgtggacggcgtggaagtgcacaacgccaagaccaagcctagagaggaacagtacaacagcacctacagagtggtgtccgtgctgacagtgctgcaccaggattggctgaacggcaaagagtacaagtgcaaggtgtccaacaaggccctgcctgctcctatcgagaaaaccatcagcaaggccaagggccagcctagggaaccccaggtttacacccttcctccatgccgggatgagctgaccaagaaccaggtgtccctgtggtgtctcgtgaagggcttctacccctccgatatcgccgtggaatgggagagcaatggccagcctgagaacaactacaagacaacccctcctgtgctggacagcgacggctcattcttcctgtacagcaagctgaccgtggacaagtccagatggcagcagggcaacgtgttcagctgctccgtgatgcacgaggccctgcacaaccactacacacagaagtccctgtctctgagccccggcaaa

SEQ ID NO: 27 - DNA, 2151 bp, Artificial
  Full-length nucleotide sequence of CX3-0002-HC_k
atgaagcacctgtggttctttctgctgctggtggccgctcctagatgggtgctgtctggacaggttcagctggttcagtctggcgccgaagtgaagaaacctggcgcctctgtgaaggtgtcctgcaaggcctctggctacgccttcagcaactacctgatcgagtgggtccgacaggcccctggacaaggacttgaatggatgggcgtgatcaaccctggcagcggcgtgaccaactacaacgagaagttcaagggcagagtgaccatcaccgccgacaccagcacaagcaccgcctacatggaactgagcagcctgagaagcgaggacaccgccgtgtactattgtgccagagccgaggcttggtttgcctattggggacagggcaccctggtcaccgttagctctggtggaggcggttcaggcggaggtggcagcggcggtggcgggagtgatattgtgatgacacagagccccgacagcctggccgtgtctcttggagaaagagccaccatcaactgcaagagcagccagagcctgctgtactccagcaaccagaagaactacctggcctggtatcagcagaagcccggccagcctcctaagctgctgatctactgggccagcaccagagaaagcggcgtgcccgatagattttctggctctggcagcggcaccgacttcaccctgacaatttctagcctgcaagccgaggacgtggccgtgtactactgccagagatattacggctacccctggacctttggccagggcaccaaggtggaaatcaagggaggcggaggatctgaggtgcagcttgttgaatcaggtggcggacttgtgcagcctggcggaagcctcagacttagctgtgctgcttccggcgtgaccttcaactactacggcatgagctggatcaggcaggcacctggaaagggcctcgagtgggttgcctctatcacaagaagcggcggcagaatctactaccccgactctgtgaaaggccggttcaccatctccagagagaacacccagaaaacactctatctccagatgaactctctgcgcgccgaagatacagccgtctattactgcaccctggacggcagagatggctgggttgcatattggggacagggaaccctcgtgaccgtgtcctctgcctctacaaagggccctagcgtgttccctctggctcctagcagcaagtctaccagcggaggaacagccgctctgggctgtctggtcaaggactactttcccgagccagtgacagtgtcctggaactctggcgctctgacatccggcgtgcacacatttccagccgtgctgcaaagctccggcctgtactctctgagcagcgtggtcacagtgccaagctctagcctgggcacccagacctacatctgcaatgtgaaccacaagcctagcaacaccaaggtcgacaagagagtggaacccaagagctgcgacaagacccacacctgtcctccatgtcctgctccagaagctgcaggcggcccttccgtgtttctgttccctccaaagcctaaggacaccctgatgatcagccggacacctgaagtgacctgcgtggtggtggatgtgtcccacgaggatcccgaagtgaagttcaattggtacgtggacggcgtggaagtgcacaacgccaagaccaagcctagagaggaacagtacaacagcacctacagagtggtgtctgtgctgacagtgctgcaccaggactggctgaacggcaaagagtacaagtgcaaggtgtccaacaaggccctgcctgctcctatcgagaaaaccatcagcaaggccaagggccagcctagggaaccccaggtttacaccctgcctccatgcagggatgagctgaccaagaaccaggtgtccctgtggtgcctggttaagggcttctacccctccgatatcgccgtggaatgggagagcaatggccagccagagaacaactacaagacaacccctcctgtgctggactccgacggctcattcttcctgtacagcaagctgaccgtggacaagagcagatggcagcagggcaacgtgttcagctgcagcgtgatgcacgaggccctgcacaaccactacacacagaagtccctgtctctgagccccggcaaa

SEQ ID NO: 28 - DNA, 2139 bp, Artificial
  Full-length nucleotide sequence of RX3-0002-HC_k
atgaagcacctgtggttctttctgctgctggtggccgctcctagatgggtgctgtctggacaggtgcagctggtgcagtctggcgccgaagtgaagaaaccaggcgccagcgtgaaggtgtcctgcaaggccagcggctacacctttaccggctactacatgcactgggtgcgccaggctccaggccagggactggaatggatgggccggatcaaccccaatagcggcggcaccaactacgcccagaaattccagggcagagtgaccatgacccgggacaccagcatcagcaccgcctacatggaactgagcggcctgagaagcgacgacaccgccgtgtactactgtgcctctggctctgtgcggcacccttggggacagggaacactcgtgaccgtgtccagcggtggaggcggttcaggcggaggtggcagcggcggtggcgggagtcagcctgtgctgacacagcctccaagcgcctctggcacacctggccagagagtgacaatcagctgcagcggcagcagaagcaacatcggcggcaacatcgtgtcctggtatcagcagttccccggcaccgcccctagactgctgacctacgccgacaaccagaggcctagcggcgtgcccgatagattcagcggctctaagagcggcaccagcgccagcctggccatctctggcctgcagtctgaggacgaggccgactactattgcgccgcctgggacgacagcctgaacggcgtggtgtttggcggaggcaccaagctgacagtgctgggaggcggaggatctgaggtgcagcttgttgaatcaggtggcggacttgtgcagcctggcggaagcctcagacttagctgtgctgcttccggcgtgaccttcaactactacggcatgagctggatcaggcaggcacctggaaagggcctcgagtgggttgcctctatcacaagaagcggcggcagaatctactaccccgactctgtgaaaggccggttcaccatctccagagagaacacccagaaaacactctatctccagatgaactctctgcgcgccgaagatacagccgtctattactgcaccctggacggcagagatggctgggttgcatattggggacagggaaccctcgtgaccgtgtcctctgcctctacaaagggccctagcgtgttccctctggctcctagcagcaagtctaccagcggaggaacagccgctctgggctgtctggtcaaggactactttcccgagccagtgacagtgtcctggaactctggcgctctgacatccggcgtgcacacatttccagccgtgctgcaaagctccggcctgtactctctgagcagcgtggtcacagtgccaagctctagcctgggcacccagacctacatctgcaatgtgaaccacaagcctagcaacaccaaggtcgacaagagagtggaacccaagagctgcgacaagacccacacctgtcctccatgtcctgctccagaagctgcaggcggcccttccgtgtttctgttccctccaaagcctaaggacaccctgatgatcagccggacacctgaagtgacctgcgtggtggtggatgtgtcccacgaggatcccgaagtgaagttcaattggtacgtggacggcgtggaagtgcacaacgccaagaccaagcctagagaggaacagtacaacagcacctacagagtggtgtctgtgctgacagtgctgcaccaggactggctgaacggcaaagagtacaagtgcaaggtgtccaacaaggccctgcctgctcctatcgagaaaaccatcagcaaggccaagggccagcctagggaaccccaggtttacaccctgcctccatgcagggatgagctgaccaagaaccaggtgtccctgtggtgcctggttaagggcttctacccctccgatatcgccgtggaatgggagagcaatggccagccagagaacaactacaagacaacccctcctgtgctggactccgacggctcattcttcctgtacagcaagctgaccgtggacaagagcagatggcagcagggcaacgtgttcagctgcagcgtgatgcacgaggccctgcacaaccactacacacagaagtccctgtctctgagccccggcaaa

SEQ ID NO: 29 - protein, 718 aa, Artificial
  Full-length amino acid sequence of TX3-0002-HC_k
MKHLWFFLLLVAAPRWVLSGQVQLVQSGAEVKKPGASVKVSCKASGYTFTTAGMQWVRQAPGQGLEWMGWINTHSGVPKYAEDFKGRVTISADTSTSTAYLQLSSLKSEDTAVYYCARSGFGSSYWYFDVWGQGTLVTVSSGGGGSGGGGSGGGGSDIQMTQSPSSLSASVGDRVTITCKASQDVSTAVAWYQQKPGKAPKLLIYSASYRYTGVPSRFSGSGSGTDFTLTISSLQPEDFAVYYCQQHYITPLTFGQGTKLEIKRTGGGGSEVQLVESGGGLVQPGGSLRLSCAASGVTFNYYGMSWIRQAPGKGLEWVASITRSGGRIYYPDSVKGRFTISRENTQKTLYLQMNSLRAEDTAVYYCTLDGRDGWVAYWGQGTLVTVSSASTKGPSVFPLAPSSKSTSGGTAALGCLVKDYFPEPVTVSWNSGALTSGVHTFPAVLQSSGLYSLSSVVTVPSSSLGTQTYICNVNHKPSNTKVDKRVEPKSCDKTHTCPPCPAPEAAGGPSVFLFPPKPKDTLMISRTPEVTCVVVDVSHEDPEVKFNWYVDGVEVHNAKTKPREEQYNSTYRVVSVLTVLHQDWLNGKEYKCKVSNKALPAPIEKTISKAKGQPREPQVYTLPPCRDELTKNQVSLWCLVKGFYPSDIAVEWESNGQPENNYKTTPPVLDSDGSFFLYSKLTVDKSRWQQGNVFSCSVMHEALHNHYTQKSLSLSPGK

SEQ ID NO: 30 - protein, 717 aa, Artificial
  Full-length amino acid sequence of CX3-0002-HC_k
MKHLWFFLLLVAAPRWVLSGQVQLVQSGAEVKKPGASVKVSCKASGYAFSNYLIEWVRQAPGQGLEWMGVINPGSGVTNYNEKFKGRVTITADTSTSTAYMELSSLRSEDTAVYYCARAEAWFAYWGQGTLVTVSSGGGGSGGGGSGGGGSDIVMTQSPDSLAVSLGERATINCKSSQSLLYSSNQKNYLAWYQQKPGQPPKLLIYWASTRESGVPDRFSGSGSGTDFTLTISSLQAEDVAVYYCQRYYGYPWTFGQGTKVEIKGGGGSEVQLVESGGGLVQPGGSLRLSCAASGVTFNYYGMSWIRQAPGKGLEWVASITRSGGRIYYPDSVKGRFTISRENTQKTLYLQMNSLRAEDTAVYYCTLDGRDGWVAYWGQGTLVTVSSASTKGPSVFPLAPSSKSTSGGTAALGCLVKDYFPEPVTVSWNSGALTSGVHTFPAVLQSSGLYSLSSVVTVPSSSLGTQTYICNVNHKPSNTKVDKRVEPKSCDKTHTCPPCPAPEAAGGPSVFLFPPKPKDTLMISRTPEVTCVVVDVSHEDPEVKFNWYVDGVEVHNAKTKPREEQYNSTYRVVSVLTVLHQDWLNGKEYKCKVSNKALPAPIEKTISKAKGQPREPQVYTLPPCRDELTKNQVSLWCLVKGFYPSDIAVEWESNGQPENNYKTTPPVLDSDGSFFLYSKLTVDKSRWQQGNVFSCSVMHEALHNHYTQKSLSLSPGK

SEQ ID NO: 31 - protein, 713 aa, Artificial
  Full-length amino acid sequence of RX3-0002-HC_k
MKHLWFFLLLVAAPRWVLSGQVQLVQSGAEVKKPGASVKVSCKASGYTFTGYYMHWVRQAPGQGLEWMGRINPNSGGTNYAQKFQGRVTMTRDTSISTAYMELSGLRSDDTAVYYCASGSVRHPWGQGTLVTVSSGGGGSGGGGSGGGGSQPVLTQPPSASGTPGQRVTISCSGSRSNIGGNIVSWYQQFPGTAPRLLTYADNQRPSGVPDRFSGSKSGTSASLAISGLQSEDEADYYCAAWDDSLNGVVFGGGTKLTVLGGGGSEVQLVESGGGLVQPGGSLRLSCAASGVTFNYYGMSWIRQAPGKGLEWVASITRSGGRIYYPDSVKGRFTISRENTQKTLYLQMNSLRAEDTAVYYCTLDGRDGWVAYWGQGTLVTVSSASTKGPSVFPLAPSSKSTSGGTAALGCLVKDYFPEPVTVSWNSGALTSGVHTFPAVLQSSGLYSLSSVVTVPSSSLGTQTYICNVNHKPSNTKVDKRVEPKSCDKTHTCPPCPAPEAAGGPSVFLFPPKPKDTLMISRTPEVTCVVVDVSHEDPEVKFNWYVDGVEVHNAKTKPREEQYNSTYRVVSVLTVLHQDWLNGKEYKCKVSNKALPAPIEKTISKAKGQPREPQVYTLPPCRDELTKNQVSLWCLVKGFYPSDIAVEWESNGQPENNYKTTPPVLDSDGSFFLYSKLTVDKSRWQQGNVFSCSVMHEALHNHYTQKSLSLSPGK

SEQ ID NO: 32 - protein, 8 aa, Artificial
  Amino acid sequence of heavy chain CDR1 of C3E-7085
GVTFNYYG

SEQ ID NO: 33 - protein, 8 aa, Artificial
  Amino acid sequence of heavy chain CDR2 of C3E-7085
ITRSGGRI

SEQ ID NO: 34 - protein, 11 aa, Artificial
  Amino acid sequence of heavy chain CDR3 of C3E-7085
TLDGRDGWVAY

SEQ ID NO: 35 - protein, 8 aa, Artificial
  Amino acid sequence of light chain CDR1 of C3E-7085
TGNIGSNY

SEQ ID NO: 36 - protein, 3 aa, Artificial
  Amino acid sequence of light chain CDR2 of C3E-7085
RDD

SEQ ID NO: 37 - protein, 8 aa, Artificial
  Amino acid sequence of light chain CDR3 of C3E-7085
QSYSSGFI

SEQ ID NO: 38 - protein, 5 aa, Artificial
  Peptide linker
GGGGS

SEQ ID NO: 39 - protein, 240 aa, Artificial
  Amino acid sequence of C3E-7097
EVQLVESGGGLVQPGGSLRLSCAASGVTFNYYGMSWIRQAPGKCLEWVASITRSGGRIYYPDSVKGRFTISRENTQKTLYLQMNSLRAEDTAVYYCTLDGRDGWVAYWGQGTLVTVSSGGGGSGGGGSGGGGSNFMLTQPSSVSGVPGQRVTISCTGNTGNIGSNYVNWYQQLPGTAPKLLIYRDDKRPSGVPDRFSGSKSGTSASLAITGFQAEDEADYYCQSYSSGFIFGCGTKLTVL

SEQ ID NO: 40 - protein, 8 aa, Artificial
  Amino acid sequence of heavy chain CDR1 of C3E-7093
GVTFNYYG

SEQ ID NO: 41 - protein, 8 aa, Artificial
  Amino acid sequence of heavy chain CDR2 of C3E-7093
ITSSGGRI

SEQ ID NO: 42 - protein, 11 aa, Artificial
  Amino acid sequence of heavy chain CDR3 of C3E-7093
TLDGRDGWVAY

SEQ ID NO: 43 - protein, 8 aa, Artificial
  Amino acid sequence of light chain CDR1 of C3E-7093
TGNIGSNY

SEQ ID NO: 44 - protein, 3 aa, Artificial
  Amino acid sequence of light chain CDR2 of C3E-7093
RND

SEQ ID NO: 45 - protein, 8 aa, Artificial
  Amino acid sequence of light chain CDR3 of C3E-7093
QSYSSGFI

SEQ ID NO: 46 - protein, 216 aa, Artificial
  Amino acid sequence of C3E-7093-Fab
EVQLVESGGGLVQPGGSLRLSCAASGVTFNYYGMSWIRQAPGKGLEWVASITSSGGRIYYPDSVKGRFTISRENTQKTLYLQMNSLRAEDTAVYYCTLDGRDGWVAYWGQGTLVTVSSASTKGPSVFPLAPSSKSTSGGTAALGCLVKDYFPEPVTVSWNSGALTSGVHTFPAVLQSSGLYSLSSVVTVPSSSLGTQTYICNVNHKPSNTKVDKRV

SEQ ID NO: 47 - protein, 215 aa, Artificial
  Amino acid sequence of C3E-7093-LC
NFMLTQPHSVSESPGKTVTISCKRNTGNIGSNYVNWYQQHEGSSPTTIIYRNDKRPDGVSDRFSGSIDRSSKSASLTISNLKTEDEADYFCQSYSSGFIFGGGTKLTVLGQPKAAPSVTLFPPSSEELQANKATLVCLISDFYPGAVTVAWKADSSPVKAGVETTTPSKQSNNKYAASSYLSLTPEQWKSHRSYSCQVTHEGSTVEKTVAPTECS

SEQ ID NO: 48 - protein, 242 aa, Artificial
  Amino acid sequence of C3E-7098
EVQLVESGGGLVQPGGSLRLSCAASGVTFNYYGMSWIRQAPGKGLEWVASITSSGGRIYYPDSVKGRFTISRENTQKTLYLQMNSLRAEDTAVYYCTLDGRDGWVAYWGCGTLVTVSSGGGGSGGGGSGGGGSNFMLTQPHSVSESPGKTVTISCKRNTGNIGSNYVNWYQQHEGSCPTTIIYRNDKRPDGVSDRFSGSIDRSSKSASLTISNLKTEDEADYFCQSYSSGFIFGGGTKLTVL

SEQ ID NO: 49 - protein, 242 aa, Artificial
  Amino acid sequence of C3E-7099
EVQLVESGGGLVQPGGSLRLSCAASGVTFNYYGMSWIRQAPGKCLEWVASITSSGGRIYYPDSVKGRFTISRENTQKTLYLQMNSLRAEDTAVYYCTLDGRDGWVAYWGQGTLVTVSSGGGGSGGGGSGGGGSNFMLTQPHSVSESPGKTVTISCKRNTGNIGSNYVNWYQQHEGSSPTTIIYRNDKRPDGVSDRFSGSIDRSSKSASLTISNLKTEDEADYFCQSYSSGFIFGCGTKLTVL